European Patent Application EP 4 477 666 A1, published December 18, 2024. Title: Anti-NPC VHH antibodies and methods for their stabilization. Applicant: Max-Planck-Gesellschaft zur Foerderung der Wissenschaften e.V. The sequence listing filed with the application follows.

SEQUENCE LISTING (45 sequences)

SEQ ID NO: 1 - protein, 123 aa, synthetic construct
  REGION 1..123: note = VHH antibody sequence, KG1D08
QVQLVESGGGLVQAGGSLRLSCAASGRSFRGNIMAWFRQTPGKERLFVASITGSGYTSYENSVKGRFTISRDSARDTVDLQMTTLAPEDTAVYYCAGRFRGGHNRMPDAYEYWGQGTQVTVSS

SEQ ID NO: 2 - protein, 13 aa, synthetic construct
  REGION 1..13: note = CDR1_KG1D08
AASGRSFRGNIMA

SEQ ID NO: 3 - protein, 14 aa, synthetic construct
  REGION 1..14: note = CDR2_KG1D08
ASITGSGYTSYENS

SEQ ID NO: 4 - protein, 17 aa, synthetic construct
  REGION 1..17: note = CDR3_KG1D08
AGRFRGGHNRMPDAYEY

SEQ ID NO: 5 - protein, 120 aa, synthetic construct
  REGION 1..120: note = VHH antibody sequence, KG1C05
QVQLVESGGGLVQAGGSLRLACATSGILLSKAVMDWYRQIPGKQRELVARTGIRDSATYADFVKGRFTVSRENENNTVYLQMNSLQPEDAGLYVCKAAVTGVFGRLSEHWGQGTQVTVSS

SEQ ID NO: 6 - protein, 13 aa, synthetic construct
  REGION 1..13: note = CDR1_KG1C05
ATSGILLSKAVMD

SEQ ID NO: 7 - protein, 14 aa, synthetic construct
  REGION 1..14: note = CDR2_KG1C05
ARTGIRDSATYADF

SEQ ID NO: 8 - protein, 14 aa, synthetic construct
  REGION 1..14: note = CDR3_KG1C05
KAAVTGVFGRLSEH

SEQ ID NO: 9 - protein, 119 aa, synthetic construct
  REGION 1..119: note = VHH antibody sequence, KG2E04
QVQLVESGGGLVQAGGSLRLSCAASGRGFSGYTWGWFRQVPGKDRTFVAAMSWITGSTYYADSVKGRFTISGDNAKNTLLLQMDNLKPNDTAVYYCAARSKVSPDYDIWGQGTQVTVSS

SEQ ID NO: 10 - protein, 13 aa, synthetic construct
  REGION 1..13: note = CDR1_KG2E04
AASGRGFSGYTWG

SEQ ID NO: 11 - protein, 15 aa, synthetic construct
  REGION 1..15: note = CDR2_KG2E04
AAMSWITGSTYYADS

SEQ ID NO: 12 - protein, 12 aa, synthetic construct
  REGION 1..12: note = CDR3_KG2E04
AARSKVSPDYDI

SEQ ID NO: 13 - protein, 119 aa, synthetic construct
  REGION 1..119: note = VHH antibody sequence, KG2B08
QVQLVESGGGLVQAGGSLRLSCAASGRGFSGYTWGWFRQVPGKERTFVAAMSWITGSTYYADSVKGRFTISGDNAKNTLLLQMNNLKPGDTAVYYCAARSKVSYDYDIWGQGTQVTVSS

SEQ ID NO: 14 - protein, 13 aa, synthetic construct
  REGION 1..13: note = CDR1_KG2B08
AASGRGFSGYTWG

SEQ ID NO: 15 - protein, 15 aa, synthetic construct
  REGION 1..15: note = CDR2_KG2B08
AAMSWITGSTYYADS

SEQ ID NO: 16 - protein, 12 aa, synthetic construct
  REGION 1..12: note = CDR3_KG2B08
AARSKVSYDYDI

SEQ ID NO: 17 - protein, 119 aa, synthetic construct
  REGION 1..119: note = VHH antibody sequence, KG2B12
QVQLVESGGGLVQAGGSLRLSCAASGRGFSGYTWGWFRQVPGKERTFVAAMSWITGSTYYADSVKGRFTISGDNAKNTLLLQMNNLKPGDTAVYYCAARSKVSYDYDIWGQGTLVTVSS

SEQ ID NO: 18 - protein, 13 aa, synthetic construct
  REGION 1..13: note = CDR1_KG2B12
AASGRGFSGYTWG

SEQ ID NO: 19 - protein, 15 aa, synthetic construct
  REGION 1..15: note = CDR2_KG2B12
AAMSWITGSTYYADS

SEQ ID NO: 20 - protein, 12 aa, synthetic construct
  REGION 1..12: note = CDR3_KG2B12
AARSKVSYDYDI

SEQ ID NO: 21 - protein, 115 aa, synthetic construct
  REGION 1..115: note = VHH antibody sequence, Re3E01
QVQLVESGGGLVQPGGSLRLSCAASGFTFTDYLMAWYRQAPGNQRQLVAYITSDGSTVYASSARGRFTISRDNAKNTVTLQMNSLLLDDTAVYYCSAKSGLKDYYGQGTQVTVSS

SEQ ID NO: 22 - protein, 13 aa, synthetic construct
  REGION 1..13: note = CDR1_Re3E01
AASGFTFTDYLMA

SEQ ID NO: 23 - protein, 14 aa, synthetic construct
  REGION 1..14: note = CDR2_Re3E01
AYITSDGSTVYASS

SEQ ID NO: 24 - protein, 9 aa, synthetic construct
  REGION 1..9: note = CDR3_Re3E01
SAKSGLKDY

SEQ ID NO: 25 - protein, 128 aa, synthetic construct
  REGION 1..128: note = VHH antibody sequence, xhNup358-Nb2t MS41
QVQLVESGGGLVQPGGSLRLSCAASGRPLSDYAMGWFRQAPGKEREFVAAISWKGGETFYAGSVKGRFTISRDDAKNSLYLQMNNLKLEDTAEYSCAAVLGSPHYSGTHYYPAEYDYWGQGTQVTVSS

SEQ ID NO: 26 - protein, 13 aa, synthetic construct
  REGION 1..13: note = CDR1_xhNup358-Nb2t
AASGRPLSDYAMG

SEQ ID NO: 27 - protein, 15 aa, synthetic construct
  REGION 1..15: note = CDR2_xhNup358-Nb2t
AAISWKGGETFYAGS

SEQ ID NO: 28 - protein, 21 aa, synthetic construct
  REGION 1..21: note = CDR3_xhNup358-Nb2t
AAVLGSPHYSGTHYYPAEYDY

SEQ ID NO: 29 - protein, 129 aa, synthetic construct
  REGION 1..129: note = VHH antibody sequence, xhNup93-Nb3t MS25
QVQLVESGGGVVQTGDSLMLSCLFSGRPGRVFGHYLMGWFRQIPGKERDVVAAISFSGDPTYYADSVKGRATISRDNAKNTVYLQMNGLKSEDTAVYYCAADRLPYGDSWASKDEYDYWGQGTQVTVSS

SEQ ID NO: 30 - protein, 16 aa, synthetic construct
  REGION 1..16: note = CDR1_xhNup93-Nb3t
LFSGRPGRVFGHYLMG

SEQ ID NO: 31 - protein, 15 aa, synthetic construct
  REGION 1..15: note = CDR2_xhNup93-Nb3t
AAISFSGDPTYYADS

SEQ ID NO: 32 - protein, 19 aa, synthetic construct
  REGION 1..19: note = CDR3_xhNup93-Nb3t
AADRLPYGDSWASKDEYDY

SEQ ID NO: 33 - protein, 120 aa, synthetic construct
  REGION 1..120: note = VHH antibody sequence, xhNup35-Nb1t
QVQLVESGGGLVQAGGSLRLSCVGTGNISSAYTMAWYRQAAGKEREVVAGILNGGSTHYADSVKGRFTISRDNAKNTVYLQMNSLQPEDTGVYCCHVVIESTRFVYDHYWGQGTRVTVSS

SEQ ID NO: 34 - protein, 13 aa, synthetic construct
  REGION 1..13: note = CDR1_xhNup35-Nb1t
VGTGNISSAYTMA

SEQ ID NO: 35 - protein, 14 aa, synthetic construct
  REGION 1..14: note = CDR2_xhNup35-Nb1t
AGILNGGSTHYADS

SEQ ID NO: 36 - protein, 14 aa, synthetic construct
  REGION 1..14: note = CDR3_xhNup35-Nb1t
HVVIESTRFVYDHY

SEQ ID NO: 37 - protein, 115 aa, synthetic construct
  REGION 1..115: note = VHH antibody sequence, Nb116
QVQLVESGGGLVQPGGSLTLSCTVSRIINWTRMGWSRTAPGKQREFVANIDPSGTTNYADFVKGRFAISVNNDKRTVFLQMNGLKPEDTAVYRCFTIEPDRGTNWGQGTQVTVSS

SEQ ID NO: 38 - protein, 12 aa, synthetic construct
  REGION 1..12: note = CDR1_Nb116
TVSRIINWTRMG

SEQ ID NO: 39 - protein, 14 aa, synthetic construct
  REGION 1..14: note = CDR2_Nb116
ANIDPSGTTNYADF

SEQ ID NO: 40 - protein, 10 aa, synthetic construct
  REGION 1..10: note = CDR3_Nb116
FTIEPDRGTN

SEQ ID NO: 41 - protein, 189 aa, Escherichia coli
  REGION 1..189: note = protein disulfide isomerase DsbA
AQYEDGKQYTTLEKPVAGAPQVLEFFSFFCPHCYQFEEVLHISDNVKKKLPEGVKMTKYHVNFMGGDLGKDLTQAWAVAMALGVEDKVTVPLFEGVQKTQTIRSASDIRDVFINAGIKGEEYDAAWNSFVVKSLVAQQEKAAADVQLRGVPAMFVNGKYQLNPQGMDTSNMDVFVQQYADTVKYLSEKK

SEQ ID NO: 42 - protein, 216 aa, Escherichia coli
  REGION 1..216: note = protein disulfide isomerase DsbC
DDAAIQQTLAKMGIKSSDIQPAPVAGMKTVLTNSGVLYITDDGKHIIQGPMYDVSGTAPVNVTNKMLLKQLNALEKEMIVYKAPQEKHVITVFTDITCGYCHKLHEQMADYNALGITVRYLAFPRQGLDSDAEKEMKAIWCAKDKNKAFDDVMAGKSVAPASCDVDIADHYALGVQLGVSGTPAVVLSNGTLVPGYQPPKEMKEFLDEHQKMTSGK

SEQ ID NO: 43 - protein, 232 aa, Escherichia coli
  REGION 1..232: note = protein disulfide isomerase DsbG
AEELPAPVKAIEKQGITIIKTFDAPGGMKGYLGKYQDMGVTIYLTPDGKHAISGYMYNEKGENLSNTLIEKEIYAPAGREMWQRMEQSHWLLDGKKDAPVIVYVFADPFCPYCKQFWQQARPWVDSGKVQLRTLLVGVIKPESPATAAAILASKDPAKTWQQYEASGGKLKLNVPANVSTEQMKVLSDNEKLMDDLGANVTPAIYYMSKENTLQQAVGLPDQKTLNIIMGNK

SEQ ID NO: 44 - protein, 130 aa, synthetic construct
  REGION 1..130: note = VHH antibody sequence, Re9B09
QVQLVESGGGLVQPGGSLRLSCAASGFTLDYYAIGWFRQAPGKEREGVSRISSSDGSTDYADSVKGRFTISRDNAKNTVYLQMNSLKPEDTAVYYCATVPGTYYSGNWYYTWHPEAVDYWGKGTQVTVSS

SEQ ID NO: 45 - protein, 127 aa, synthetic construct
  REGION 1..127: note = VHH antibody sequence, Re24H12
QVQLVESGGGLVQPGGSLRLSCAASGFTLDYYAIGWFRQAPGKEREGVSYIRSSDGTTYYADSVKGRFTISRDNAKNTVYLQMNSLKPEDTAVYYCAADEAYYSELGWESPWGWSYWGQGTQVTVSS